European Patent Application EP 4 574 987 A1, published June 25, 2025. Title: Verfahren zur Herstellung von 2,5-Furandicarbonsäure. Applicant: Annikki GmbH. The sequence listing filed with the application follows.

SEQUENCE LISTING (10 sequences)

SEQ ID NO: 1 - DNA, 1410 bp, Pseudomonas nitroreducens
  source 1..1410: mol_type = genomic DNA
atgtcacgctatgaactgctgatcgatggtcgcctgcaggcggccgagcactacgaccgggtgatcgacccggccagcgaagaaatcgttggcgaagccgcccgcgccagcctggagcaggtcgacgcggcggtggatgccgcacaccgcgccttcccggcctgggccaccgatctcgacgtccgccgccagagcctggcccgagccgccgaacgagtacgcgagaatgcccaggcgctggccgagctgatcacccgcgaacagggtcgcccactgcgctcgaccctggaggaagtggctggcgtcgccgccactttcgagcaccacgcgcagctggagctacccgccgacacccagttgcgcgacgacggcgagcgcctggtgcgcatcacccgcaaaccgctgggggtggtcgccgcgatcaccccgtggaacgtcccgctgatcctgctggtattgaagatcgcgcctgccctgcacgccggcaacaccgtggtggccaagccctcggagcacacgccgctgtctaccctgctgctggcgcgactgctgggcgatgtgttccccgctggcgtgttcaacgtggttgccggtgcgggcgaggttggcgaacacctggtacgtcatccgcgggtgcgccacgtgaccttcaccggcagcgtcgccaccggcaagcgcctgtatgccggcgcgggggacgacctcaagcgtcttaccctggaactgggcggcaacgacgccgcgctggtactggaagacgccgacctcgacgccatcgtcgaaccgctgttctggggcgccttctggaacagcggccaggtgtgctttgcgatcaagcgcctgtacgtgcatgacagcctgttcgaaccgttactggcgaaactcgccgagcgcgcccagcgcacccgcctcggtcatgggctcgacccgcagacggaactggggccgctgaccaacgcacagcaactggaacgggtcatcgccctggtggaagacgccaaggctcacggagcacgcatccgcagcggcggcgtacggcccgacggtcccggctacttctacccgccgaccctggtcagcggcgtggcggccggcgtcgcgctggtggacgaggaacagttcggcccggtgttgccggtgatctccttccgcaacgaagaggacgccattacccaggccaacgccagccactacggcctcggcgcctcggtgtggacccgcgacctggcgcgcggcgaagccatcgccaggcggctggaggcgggcctggcctgggtcaaccagcacggccacatccagcccggcgcgcccaagggcgggcacaagtggagcgggctcggctacgaaggcgggcagcgcggctatgaggccttcagcgagctgcaggtgctgaacatttcgcggcgctaa

SEQ ID NO: 2 - protein, 469 aa, Pseudomonas nitroreducens
MSRYELLIDGRLQAAEHYDRVIDPASEEIVGEAARASLEQVDAAVDAAHRAFPAWATDLDVRRQSLARAAERVRENAQALAELITREQGRPLRSTLEEVAGVAATFEHHAQLELPADTQLRDDGERLVRITRKPLGVVAAITPWNVPLILLVLKIAPALHAGNTVVAKPSEHTPLSTLLLARLLGDVFPAGVFNVVAGAGEVGEHLVRHPRVRHVTFTGSVATGKRLYAGAGDDLKRLTLELGGNDAALVLEDADLDAIVEPLFWGAFWNSGQVCFAIKRLYVHDSLFEPLLAKLAERAQRTRLGHGLDPQTELGPLTNAQQLERVIALVEDAKAHGARIRSGGVRPDGPGYFYPPTLVSGVAAGVALVDEEQFGPVLPVISFRNEEDAITQANASHYGLGASVWTRDLARGEAIARRLEAGLAWVNQHGHIQPGAPKGGHKWSGLGYEGGQRGYEAFSELQVLNISRR

SEQ ID NO: 3 - DNA, 1437 bp, Saccharolobus solfataricus
  source 1..1437: mol_type = genomic DNA
atgaaatcgtatcagggattggctgacaagtggattaagggcagtggggaagaataccttgatattaatccggctgataaggatcacgtattagctaagataagattatatacaaaagatgacgttaaagaagctataaacaaggctgtagccaaattcgacgaatggtcaaggactccagcacctaaaagaggctcaatattacttaaggcaggggaattaatggaacaagaagcccaagagtttgcgctattgatgacattagaggagggtaagactctcaaggatagtatgtttgaagtgacaagaagttataatttactgaaattttatggagcattagcatttaagatatctgggaaaacgcttccttcagcagatcctaatactaggatatttacagtaaaggaacccttaggcgtagtagctttaattacgccgtggaatttcccattatcaataccagtatggaaattggctccagccttggctgcgggtaacactgcagtaataaaaccagcgacgaaaacaccgttaatggtagccaaattggtagaagtgttgtctaaagctggattgccagagggtgtcgtgaatttagtagttggtaagggaagtgaagtcggagataccatagtaagtgatgataatatagctgcagtatcatttactggatcaaccgaggtaggtaagagaatttacaaactcgtaggaaataaaaatagaatgacaagaattcaactagagctaggaggtaaaaacgcgttatatgtggataagagcgctgacttaacgttagctgctgaattagccgtaagaggaggatttggactaaccggtcaatcatgtactgcaactagtaggttaataattaacaaggatgtatatactcaatttaaacaaagactactagaaagagttaagaagtggagagtaggaccgggtactgaagatgttgatatgggtccagttgtagatgaaggtcaatttaagaaagacttagaatatatagaatacggaaagaatgtgggagcaaaactaatttatggtggaaatataataccagggaagggatatttcctagaacctacaattttcgaaggagtcacatctgatatgaggctatttaaagaagagattttcggtccagtacttagtgtcactgaggcaaaagatttagatgaggctataaggctagttaacgctgtagactatggacatacagctggaatagtcgcaagcgatatcaaggcgattaacgagttcgttagtagggtagaggcaggagttataaaggttaataagccaacagtcggactggaattgcaagcaccatttggtggttttaagaattctggagccactacgtggaaagagatgggagaagatgctttagagttctaccttaaggagaagacagtatacgaaggctggtaa

SEQ ID NO: 4 - protein, 478 aa, Saccharolobus solfataricus
MKSYQGLADKWIKGSGEEYLDINPADKDHVLAKIRLYTKDDVKEAINKAVAKFDEWSRTPAPKRGSILLKAGELMEQEAQEFALLMTLEEGKTLKDSMFEVTRSYNLLKFYGALAFKISGKTLPSADPNTRIFTVKEPLGVVALITPWNFPLSIPVWKLAPALAAGNTAVIKPATKTPLMVAKLVEVLSKAGLPEGVVNLVVGKGSEVGDTIVSDDNIAAVSFTGSTEVGKRIYKLVGNKNRMTRIQLELGGKNALYVDKSADLTLAAELAVRGGFGLTGQSCTATSRLIINKDVYTQFKQRLLERVKKWRVGPGTEDVDMGPVVDEGQFKKDLEYIEYGKNVGAKLIYGGNIIPGKGYFLEPTIFEGVTSDMRLFKEEIFGPVLSVTEAKDLDEAIRLVNAVDYGHTAGIVASDIKAINEFVSRVEAGVIKVNKPTVGLELQAPFGGFKNSGATTWKEMGEDALEFYLKEKTVYEGW

SEQ ID NO: 5 - DNA, 1410 bp, Methylovorus glucosotrophus
  source 1..1410: mol_type = genomic DNA
atgtcgacatttcatttacttattgatggccatctgcaagccagtgaccaatccgatgtggtgatcaaccccgcgaccgagctggaagtcgggcgtgccccacgtgccagcgccacccaggtcgaccaggcagtggaagccgcacatcaggcatttcatcgctgggcatcacagcctgaggtgcgccagcaggcactgctgggcgcggccgccgccattcgccagcatgccgatgccctggcacgcctgatcacgcaagagcaggggcggccattgcactttacccagggcgaggtggccggggctgctgctacctttgaacactatgccgggtttgccgcgccatcggatgtggtgctgcagcaggacgaacaaaagcgggtcagcattgagcgcaggccgtttggcgtagtggctgccattacgccctggaatgtgcccatcatcctgctggtactgaaaatcgccccggccttgaaggctggcaataccgtggtcgccaagccatcggaatacaccccgctttctaccttgtacctgggtgaaattctgaaagatgtatttccgcccggcgtgctgaacgtgatagccggtgacggtcaggtgggggcgcgcctggcatcgcatccgctggtgcagaaggtgacgttcaccggcagcgtggcaaccggaaaaaaactctatgccagcgccgcgcaggatgtaaaacgcctgacgctggaactgggcggtaacgatgcggccatcgtgctggacgatgccaatgtcgatgccattgccgagaagattttctggggcgccttctggaatagcggtcaggtgtgctttgccatcaagcgcctctatgtgcacgagcgtgttttccagcccttgctcgatgccctggtgaaacgcgcgcaaaaaacccgcgtgggcgatggccagctgccgggtaccgagctggggccgcttaccaacaaagcccagtttgagcgcgtgatatcgctggtggaagacgccagacgccatggcgccaccattcattcaggcggtgctgcattgcctggccccggctatttctatccgcccaccctggtcaccggcataggcgcaggtgtcgcgctggtggatgaagagcagttcggaccagtattgccgctgattcctttccgtgatgagcaagaggcggtgcgtcaggccaacgacagtccgtttggtctgggcgcttcggtttggaccgccaatcccgaacgcggcctggcgctggtacgccagctccaggccgggctcgcctgggtcaaccagcatggcgatatccatcccggtgcgcccaagggcggctacaaatccagtggccttggctacgagggcgggctgcgtggctatgacgagttcagcgagctgcaagtcgtcaatgcggcgctggtttaa

SEQ ID NO: 6 - protein, 469 aa, Methylovorus glucosotrophus
MSTFHLLIDGHLQASDQSDVVINPATELEVGRAPRASATQVDQAVEAAHQAFHRWASQPEVRQQALLGAAAAIRQHADALARLITQEQGRPLHFTQGEVAGAAATFEHYAGFAAPSDVVLQQDEQKRVSIERRPFGVVAAITPWNVPIILLVLKIAPALKAGNTVVAKPSEYTPLSTLYLGEILKDVFPPGVLNVIAGDGQVGARLASHPLVQKVTFTGSVATGKKLYASAAQDVKRLTLELGGNDAAIVLDDANVDAIAEKIFWGAFWNSGQVCFAIKRLYVHERVFQPLLDALVKRAQKTRVGDGQLPGTELGPLTNKAQFERVISLVEDARRHGATIHSGGAALPGPGYFYPPTLVTGIGAGVALVDEEQFGPVLPLIPFRDEQEAVRQANDSPFGLGASVWTANPERGLALVRQLQAGLAWVNQHGDIHPGAPKGGYKSSGLGYEGGLRGYDEFSELQVVNAALV

SEQ ID NO: 7 - DNA, 1356 bp, Carnobacterium divergens
  source 1..1356: mol_type = genomic DNA
atgaaagtagtagtagtaggctgtacacatgcaggaacagcggcagttaagacgattttaaatgaacatccagatgcatcagtatcagtatatgagcgtaatgacaatgtctcatttctatcttgtgggattgcgttgtatgttggtggagttgtgaaagatcctgcaggtttgttttattcaagtccagaagaacttgcatcaatgggcgcgaaaattaacatggaacacaatgtgaaaaatatagataatgagaataaggtcgtagtaattgagaatttaaaaacaggcgaaacatttgaagaaagctatgataagttggtaatgacaactggatcatggccaattattcctccaattgatggaatcaatagtgaaaatattcttttgtgtaaaaactataaccaagcaaatgaaattattaaagaatcaaaaaatgctaaaaagattgtcattgttggtggtggctatattggaattgaattagttgaggcatttgcagaatctggcaagcaagtgacgctagttgatggattagatcgtattttaaacaaatatttagatgctgaattcacttctgttttagagcatgatttacaagaaagaggcgttacgctagctttaaaccaaaccgtcgagaaatttgttgccaatgaatcaggtgctgtgacagctgtgaaaacaccagttggagaatatgaggctgatttagttattttatgtgttggatttaaaccaaatactgatttgttgaaggataaagtagagatgttgccaaatggtgccatcgtagtggatgaatatatgagaacaagcgatgaagcgatttttgctgctggcgatagttgcgcggttcattataatccaactggaggctctgcgtatattccgttagctacaaatgcagttagaatgggagctttagttgggaaaaatattgtttctccaacagttaaatatcgtggcacgcaagcaacttctggtttatatttatttggttttaatataggttcaaccggattgactgaaaatagcgctcctcattttggcgtagaggttcgttcagtagttgtagaagataattatcgtccagagtttatgccgacaacagagaaagtaacgatgaaattagtttatgaagtaggaacgaatcggattgttggaggtcaaatcatgtcaaaatatgatgtgacacaatctgccaatacgttatctttatgtgttcaaaataaaatgacgattgaggatttggcttatgtagatttcttcttccaacctcactttgatcgtccttggaactatttaaatattttagcgcaagcagctgttgagcaagagcgtaaactagcaaaataa

SEQ ID NO: 8 - protein, 451 aa, Carnobacterium divergens
MKVVVVGCTHAGTAAVKTILNEHPDASVSVYERNDNVSFLSCGIALYVGGVVKDPAGLFYSSPEELASMGAKINMEHNVKNIDNENKVVVIENLKTGETFEESYDKLVMTTGSWPIIPPIDGINSENILLCKNYNQANEIIKESKNAKKIVIVGGGYIGIELVEAFAESGKQVTLVDGLDRILNKYLDAEFTSVLEHDLQERGVTLALNQTVEKFVANESGAVTAVKTPVGEYEADLVILCVGFKPNTDLLKDKVEMLPNGAIVVDEYMRTSDEAIFAAGDSCAVHYNPTGGSAYIPLATNAVRMGALVGKNIVSPTVKYRGTQATSGLYLFGFNIGSTGLTENSAPHFGVEVRSVVVEDNYRPEFMPTTEKVTMKLVYEVGTNRIVGGQIMSKYDVTQSANTLSLCVQNKMTIEDLAYVDFFFQPHFDRPWNYLNILAQAAVEQERKLAK

SEQ ID NO: 9 - DNA, 1374 bp, Streptococcus mutans
  source 1..1374: mol_type = genomic DNA
atgagcaaaattgttatcgtgggtgcaaatcatgcaggcaccgcagcaattaataccattctggataattatggcagcgaaaatgaagtggttgtgtttgatcagaatagcaacattagctttctgggttgtggtatggcactgtggattggtaaacaaattagcggtccgcagggtctgttttatgcagataaagaaagcctggaagcaaaaggtgccaaaatctatatggaaagtccggttaccgccattgattatgatgcaaaacgtgttaccgcactggttaatggtcaagaacatgttgaaagctacgagaaactgattctggcaaccggtagcaccccgattctgcctccgattaaaggtgcagccattaaagaaggtagtcgcgattttgaagcaaccctgaaaaatctgcagttcgtgaaactgtatcagaatgccgaagatgtgattaacaaactgcaggataaaagccagaatctgaatcgtattgcagttgttggtgcaggttatattggtgttgaactggcagaagcatttaaacgtctgggtaaagaagtgattctgattgacgttgttgatacctgtctggcaggttattatgatcaggatctgagcgaaatgatgcgtcagaatctggaagatcatggtatcgaactggcatttggtgaaaccgttaaagcaattgaaggtgatggtaaagtggaacgtattgttaccgataaagcaagccatgatgtggatatggttattctggcagttggttttcgtccgaatacagcactgggtaatgcaaaactgaaaacctttcgtaatggtgcctttctggtggataaaaaacaagaaaccagcatcccggatgtttatgcaattggtgattgtgcaaccgtgtatgataatgccattaacgacaccaactatattgcactggcaagcaatgcactgcgtagcggtattgttgcaggtcataatgcagccggtcataaactggaaagtctgggtgttcagggtagcaatggtatttcaatttttggcctgaatatggttagcaccggtctgacccaagaaaaagccaaacgttttggttataatccggaagttaccgcctttaccgattttcagaaagccagctttatcgagcatgataactatccggttacgctgaaaattgtgtatgacaaagatagccgtctggttctgggtgcacagatggccagcaaagaagatatgagcatgggtattcacatgtttagcctggccattcaagagaaagttaccattgaacgtctggccctgctggattatttctttctgccgcattttaatcagccgtacaactatatgaccaaagcagcactgaaagccaaataa

SEQ ID NO: 10 - protein, 457 aa, Streptococcus mutans
MSKIVIVGANHAGTAAINTILDNYGSENEVVVFDQNSNISFLGCGMALWIGKQISGPQGLFYADKESLEAKGAKIYMESPVTAIDYDAKRVTALVNGQEHVESYEKLILATGSTPILPPIKGAAIKEGSRDFEATLKNLQFVKLYQNAEDVINKLQDKSQNLNRIAVVGAGYIGVELAEAFKRLGKEVILIDVVDTCLAGYYDQDLSEMMRQNLEDHGIELAFGETVKAIEGDGKVERIVTDKASHDVDMVILAVGFRPNTALGNAKLKTFRNGAFLVDKKQETSIPDVYAIGDCATVYDNAINDTNYIALASNALRSGIVAGHNAAGHKLESLGVQGSNGISIFGLNMVSTGLTQEKAKRFGYNPEVTAFTDFQKASFIEHDNYPVTLKIVYDKDSRLVLGAQMASKEDMSMGIHMFSLAIQEKVTIERLALLDYFFLPHFNQPYNYMTKAALKAK